European Patent Application EP 4 516 812 A1, published March 5, 2025. Title: ANTI-WARS1 ANTIBODY AND USE THEREOF. Applicant: 주식회사 미림진. Application KR. The sequence listing filed with the application follows.

SEQUENCE LISTING (153 sequences)

SEQ ID NO: 1 - protein, 19 aa, synthetic construct
  REGION 1..19: note = signal peptide
MGWSYIILFLVATAADVHS

SEQ ID NO: 2 - protein, 30 aa, synthetic construct
  REGION 1..30: note = FR1 of variable region in heavy chain
EVQLLESGGGLVQPGGSLRLSCAASGFTFS

SEQ ID NO: 3 - protein, 5 aa, synthetic construct
  REGION 1..5: note = CDR1 of variable region in heavy chain
SYDMS

SEQ ID NO: 4 - protein, 14 aa, synthetic construct
  REGION 1..14: note = FR2 of variable region in heavy chain
WVRQAPGKGLEWVS

SEQ ID NO: 5 - protein, 17 aa, synthetic construct
  REGION 1..17: note = CDR2 of variable region in heavy chain
AISSGGSSIYYADSVKG

SEQ ID NO: 6 - protein, 32 aa, synthetic construct
  REGION 1..32: note = FR3 of variable region in heavy chain
RFTISRDNSKNTLYLQMNSLRAEDTAVYYCAR

SEQ ID NO: 7 - protein, 12 aa, synthetic construct
  REGION 1..12: note = CDR3 of variable region in heavy chain
DVAWDMLGDFDY

SEQ ID NO: 8 - protein, 11 aa, synthetic construct
  REGION 1..11: note = FR4 of variable region in heavy chain
WGQGTLVTVSS

SEQ ID NO: 9 - protein, 121 aa, synthetic construct
  REGION 1..121: note = variable region in heavy chain
EVQLLESGGGLVQPGGSLRLSCAASGFTFSSYDMSWVRQAPGKGLEWVSAISSGGSSIYYADSVKGRFTISRDNSKNTLYLQMNSLRAEDTAVYYCARDVAWDMLGDFDYWGQGTLVTVSS

SEQ ID NO: 10 - protein, 98 aa, synthetic construct
  REGION 1..98: note = constant region in heavy chain (CH1)
ASTKGPSVFPLAPSSKSTSGGTAALGCLVKDYFPEPVTVSWNSGALTSGVHTFPAVLQSSGLYSLSSVVTVPSSSLGTQTYICNVNHKPSNTKVDKKV

SEQ ID NO: 11 - protein, 22 aa, synthetic construct
  REGION 1..22: note = FR1 of variable region in light chain
QSVLTQPPSASGTPGQRVTISC

SEQ ID NO: 12 - protein, 13 aa, synthetic construct
  REGION 1..13: note = CDR1 of variable region in light chain
TGSSSNIGSNYVY

SEQ ID NO: 13 - protein, 15 aa, synthetic construct
  REGION 1..15: note = FR2 of variable region in light chain
WYQQLPGTAPKLLIY

SEQ ID NO: 14 - protein, 7 aa, synthetic construct
  REGION 1..7: note = CDR2 of variable region in light chain of GKB101
ANSHRPS

SEQ ID NO: 15 - protein, 32 aa, synthetic construct
  REGION 1..32: note = FR3 of variable region in light chain
GVPDRFSGSKSGTSASLAISGLRSEDEADYYC

SEQ ID NO: 16 - protein, 11 aa, synthetic construct
  REGION 1..11: note = CDR3 of variable region in light chain
GAWDDSLSAYV

SEQ ID NO: 17 - protein, 10 aa, synthetic construct
  REGION 1..10: note = FR4 of variable region in light chain
FGGGTKLTVL

SEQ ID NO: 18 - protein, 110 aa, synthetic construct
  REGION 1..110: note = variable region in light chain of GKB101
QSVLTQPPSASGTPGQRVTISCTGSSSNIGSNYVYWYQQLPGTAPKLLIYANSHRPSGVPDRFSGSKSGTSASLAISGLRSEDEADYYCGAWDDSLSAYVFGGGTKLTVL

SEQ ID NO: 19 - protein, 106 aa, synthetic construct
  REGION 1..106: note = constant light chain of GKB101
TVAAPSVFIFPPSDEQLKSGTASVVCLLNNFYPREAKVQWKVDNALQSGNSQESVTEQDSKDSTYSLSSTLTLSKADYEKHKVYACEVTHQGLSSPVTKSFNRGEC

SEQ ID NO: 20 - protein, 7 aa, synthetic construct
  REGION 1..7: note = CDR2 of variable region in light chain of S53I
ANIHRPS

SEQ ID NO: 21 - protein, 110 aa, synthetic construct
  REGION 1..110: note = variable region in light chain of S53I
QSVLTQPPSASGTPGQRVTISCTGSSSNIGSNYVYWYQQLPGTAPKLLIYANIHRPSGVPDRFSGSKSGTSASLAISGLRSEDEADYYCGAWDDSLSAYVFGGGTKLTVL

SEQ ID NO: 22 - protein, 7 aa, synthetic construct
  REGION 1..7: note = CDR2 of variable region in light chain for S53L
ANLHRPS

SEQ ID NO: 23 - protein, 110 aa, synthetic construct
  REGION 1..110: note = variable region in light chain of S53L
QSVLTQPPSASGTPGQRVTISCTGSSSNIGSNYVYWYQQLPGTAPKLLIYANLHRPSGVPDRFSGSKSGTSASLAISGLRSEDEADYYCGAWDDSLSAYVFGGGTKLTVL

SEQ ID NO: 24 - protein, 7 aa, synthetic construct
  REGION 1..7: note = CDR2 of variable region in light chain for S53T
ANTHRPS

SEQ ID NO: 25 - protein, 110 aa, synthetic construct
  REGION 1..110: note = variable region in light chain of S53T
QSVLTQPPSASGTPGQRVTISCTGSSSNIGSNYVYWYQQLPGTAPKLLIYANTHRPSGVPDRFSGSKSGTSASLAISGLRSEDEADYYCGAWDDSLSAYVFGGGTKLTVL

SEQ ID NO: 26 - protein, 7 aa, synthetic construct
  REGION 1..7: note = CDR2 of variable region in light chain for S53V
ANVHRPS

SEQ ID NO: 27 - protein, 110 aa, synthetic construct
  REGION 1..110: note = variable region in light chain of S53V
QSVLTQPPSASGTPGQRVTISCTGSSSNIGSNYVYWYQQLPGTAPKLLIYANVHRPSGVPDRFSGSKSGTSASLAISGLRSEDEADYYCGAWDDSLSAYVFGGGTKLTVL

SEQ ID NO: 28 - protein, 7 aa, synthetic construct
  REGION 1..7: note = CDR2 of variable region in light chain for S53Q
ANQHRPS

SEQ ID NO: 29 - protein, 110 aa, synthetic construct
  REGION 1..110: note = variable region in light chain of S53Q
QSVLTQPPSASGTPGQRVTISCTGSSSNIGSNYVYWYQQLPGTAPKLLIYANQHRPSGVPDRFSGSKSGTSASLAISGLRSEDEADYYCGAWDDSLSAYVFGGGTKLTVL

SEQ ID NO: 30 - protein, 7 aa, synthetic construct
  REGION 1..7: note = CDR2 of variable region in light chain for H54I
ANSIRPS

SEQ ID NO: 31 - protein, 110 aa, synthetic construct
  REGION 1..110: note = variable region in light chain of H54I
QSVLTQPPSASGTPGQRVTISCTGSSSNIGSNYVYWYQQLPGTAPKLLIYANSIRPSGVPDRFSGSKSGTSASLAISGLRSEDEADYYCGAWDDSLSAYVFGGGTKLTVL

SEQ ID NO: 32 - protein, 7 aa, synthetic construct
  REGION 1..7: note = CDR2 of variable region in light chain for H54L
ANSLRPS

SEQ ID NO: 33 - protein, 110 aa, synthetic construct
  REGION 1..110: note = variable light region in chain of H54L
QSVLTQPPSASGTPGQRVTISCTGSSSNIGSNYVYWYQQLPGTAPKLLIYANSLRPSGVPDRFSGSKSGTSASLAISGLRSEDEADYYCGAWDDSLSAYVFGGGTKLTVL

SEQ ID NO: 34 - protein, 7 aa, synthetic construct
  REGION 1..7: note = CDR2 of variable region in light chain for H54K
ANSKRPS

SEQ ID NO: 35 - protein, 110 aa, synthetic construct
  REGION 1..110: note = variable region in light chain of H54K
QSVLTQPPSASGTPGQRVTISCTGSSSNIGSNYVYWYQQLPGTAPKLLIYANSKRPSGVPDRFSGSKSGTSASLAISGLRSEDEADYYCGAWDDSLSAYVFGGGTKLTVL

SEQ ID NO: 36 - protein, 7 aa, synthetic construct
  REGION 1..7: note = CDR2 of variable region in light chain for H54Q
ANSERPS

SEQ ID NO: 37 - protein, 110 aa, synthetic construct
  REGION 1..110: note = variable region in light chain of H54Q
QSVLTQPPSASGTPGQRVTISCTGSSSNIGSNYVYWYQQLPGTAPKLLIYANSQRPSGVPDRFSGSKSGTSASLAISGLRSEDEADYYCGAWDDSLSAYVFGGGTKLTVL

SEQ ID NO: 38 - protein, 7 aa, synthetic construct
  REGION 1..7: note = CDR2 of variable region in light chain for H54F
ANSFRPS

SEQ ID NO: 39 - protein, 110 aa, synthetic construct
  REGION 1..110: note = variable region in light chain of H54F
QSVLTQPPSASGTPGQRVTISCTGSSSNIGSNYVYWYQQLPGTAPKLLIYANSFRPSGVPDRFSGSKSGTSASLAISGLRSEDEADYYCGAWDDSLSAYVFGGGTKLTVL

SEQ ID NO: 40 - protein, 7 aa, synthetic construct
  REGION 1..7: note = CDR2 of variable region in light chain for SH/IL
ANILRPS

SEQ ID NO: 41 - protein, 110 aa, synthetic construct
  REGION 1..110: note = variable region in light chain of SH/IL
QSVLTQPPSASGTPGQRVTISCTGSSSNIGSNYVYWYQQLPGTAPKLLIYANILRPSGVPDRFSGSKSGTSASLAISGLRSEDEADYYCGAWDDSLSAYVFGGGTKLTVL

SEQ ID NO: 42 - protein, 7 aa, synthetic construct
  REGION 1..7: note = CDR2 of variable region in light chain for SH/LL
ANLLRPS

SEQ ID NO: 43 - protein, 110 aa, synthetic construct
  REGION 1..110: note = variable region in light chain of SH/LL
QSVLTQPPSASGTPGQRVTISCTGSSSNIGSNYVYWYQQLPGTAPKLLIYANLLRPSGVPDRFSGSKSGTSASLAISGLRSEDEADYYCGAWDDSLSAYVFGGGTKLTVL

SEQ ID NO: 44 - protein, 7 aa, synthetic construct
  REGION 1..7: note = CDR2 of variable region in light chain for SH/QL
ANQLRPS

SEQ ID NO: 45 - protein, 110 aa, synthetic construct
  REGION 1..110: note = variable region in light chain of SH/QL
QSVLTQPPSASGTPGQRVTISCTGSSSNIGSNYVYWYQQLPGTAPKLLIYANQLRPSGVPDRFSGSKSGTSASLAISGLRSEDEADYYCGAWDDSLSAYVFGGGTKLTVL

SEQ ID NO: 46 - protein, 11 aa, synthetic construct
  REGION 1..11: note = CDR3 of variable region in light chain
GAWDDSNSAYV

SEQ ID NO: 47 - protein, 110 aa, synthetic construct
  REGION 1..110: note = variable region in light chain of SHL/ILN
QSVLTQPPSASGTPGQRVTISCTGSSSNIGSNYVYWYQQLPGTAPKLLIYANILRPSGVPDRFSGSKSGTSASLAISGLRSEDEADYYCGAWDDSNSAYVFGGGTKLTVL

SEQ ID NO: 48 - protein, 110 aa, synthetic construct
  REGION 1..110: note = variable region in light chain of SHL/LLN
QSVLTQPPSASGTPGQRVTISCTGSSSNIGSNYVYWYQQLPGTAPKLLIYANLLRPSGVPDRFSGSKSGTSASLAISGLRSEDEADYYCGAWDDSNSAYVFGGGTKLTVL

SEQ ID NO: 49 - protein, 110 aa, synthetic construct
  REGION 1..110: note = variable region in light chain of SHL/QLN
QSVLTQPPSASGTPGQRVTISCTGSSSNIGSNYVYWYQQLPGTAPKLLIYANQLRPSGVPDRFSGSKSGTSASLAISGLRSEDEADYYCGAWDDSNSAYVFGGGTKLTVL

SEQ ID NO: 50 - protein, 24 aa, synthetic construct
  REGION 1..24: note = linker
EPPKSCDKTHTCPPCPAPELLGGP

SEQ ID NO: 51 - protein, 208 aa, synthetic construct
  REGION 1..206: note = Fc region
SVFLFPPKPKDTLMISRTPEVTCVVVDVSHEDPEVKFNWYVDGVEVHNAKTKPREEQYNSTYRVVSVLTVLHQDWLNGKEYKCKVSNKALPAPIEKTISKAKGQPREPQVYTLPPSREEMTKNQVSLTCLVKGFYPSDIAVEWESNGQPENNYKTTPPVLDSDGSFFLYSKLTVDKSRWQQGNVFSCSVMHEALHNHYTQKSLSLPGK

SEQ ID NO: 52 - DNA, 1416 bp, synthetic construct
  misc_feature 1..420: note = nucleotide sequence of heavy chain conjuated with signal peptide
  source 1..1416: mol_type = other DNA
atgggatggagctatatcatcctctttttggtggccacagcggccgatgtccactcggaggtgcagctgttggagtctgggggaggcttggtacagcctggggggtccctgagactctcctgtgcagcctctggattcacctttagcagttatgatatgagctgggtccgccaggctccagggaaggggctggagtgggtctcagcgatctcttctggtggtagtagtatatattacgctgattctgtaaaaggtcggttcaccatctccagagacaattccaagaacacgctgtatctgcaaatgaacagcctgagagccgaggacacggccgtgtattactgtgcgagagatgttgcttgggatatgcttggggatttcgactactggggccagggtacactggtcaccgtgagctcagctagcaccaagggcccatcggtcttccccctggcaccctcctccaagagcacctctgggggcacagcggccctgggctgcctggtcaaggactacttccccgaaccggtgacggtgtcgtggaactcaggcgccctgaccagcggcgtgcacaccttcccggctgtcctacagtcctcaggactctactccctcagcagcgtggtgaccgtgccctccagcagcctgggcacccagacctacatctgcaacgtgaatcacaagcccagcaacaccaaggtggacaagaaagttgagccccctaaatcttgtgacaaaactcacacatgcccaccgtgcccagcacctgaactcctggggggaccgtcagtcttcctcttccccccaaaacccaaggacaccctcatgatctcccggacccctgaggtcacatgcgtggtggtggacgtgagccacgaagaccctgaggtcaagttcaactggtacgtggacggcgtggaggtgcataatgccaagacaaagccgcgggaggagcagtacaacagcacgtaccgtgtggtcagcgtcctcaccgtcctgcaccaggactggctgaatggcaaggagtacaagtgcaaggtctccaacaaagccctcccagcccccatcgagaaaaccatctccaaagccaaagggcagccccgagaaccacaggtgtacaccctgcccccatcccgggacgagctgaccaagaaccaggtcagcctgacctgcctggtcaaaggcttctatcccagcgacatcgccgtggagtgggagagcaatgggcagccggagaacaactacaagaccacgcctcccgtgctggactccgacggctccttcttcctctacagcaagctcaccgtggacaagagcaggtggcagcaggggaacgtcttctcatgctccgtgatgcatgaggctctgcacaaccactacacgcagaagagcctctccctgtctccgggtaaatga

SEQ ID NO: 53 - DNA, 711 bp, synthetic construct
  misc_feature 1..711: note = nucleotide sequence of light chain conjugated with signal peptide
  source 1..711: mol_type = other DNA
atgggatggagctatatcatcctctttttggtggccacagcggccgatgtccactcgcagtctgtgctgactcagccaccctcagcgtctgggacccccgggcagagggtcaccatctcttgtactggctcttcatctaatattggcagtaattatgtctactggtaccagcagctcccaggaacggcccccaaactcctcatctatgctaatagtcatcggccaagcggggtccctgaccgattctctggctccaagtctggcacctcagcctccctggccatcagtgggctccggtccgaggatgaggctgattattactgtggtgcttgggatgatagcctgagtgcttatgtcttcgggggaggcaccaagctgacggtcctaagatctgtggctgcaccatctgtcttcatcttcccgccatctgatgagcagttgaaatctggaactgcctctgttgtgtgcctgctgaataacttctatcccagagaggccaaagtacagtggaaggtggataacgccctccaatcgggtaactcccaggagagtgtcacagagcaggacagcaaggacagcacctacagcctcagcagcaccctgacgctgagcaaagcagactacgagaaacacaaagtctacgcctgcgaagtcacccatcagggcctgagctcgcccgtcacaaagagcttcaacaggggagagtgttag

SEQ ID NO: 54 - DNA, 711 bp, synthetic construct
  misc_feature 1..711: note = nucleotides coding light chain of S53I conjuated with signal peptide
  source 1..711: mol_type = other DNA
atgggatggagctatatcatcctctttttggtggccacagcggccgatgtccactcgcagtctgtgctgactcagccaccctcagcgtctgggacccccgggcagagggtcaccatctcttgtactggctcttcatctaatattggcagtaattatgtctactggtaccagcagctcccaggaacggcccccaaactcctcatctatgctaatattcatcggccaagcggggtccctgaccgattctctggctccaagtctggcacctcagcctccctggccatcagtgggctccggtccgaggatgaggctgattattactgtggtgcttgggatgatagcctgagtgcttatgtcttcgggggaggcaccaagctgacggtcctaagatctgtggctgcaccatctgtcttcatcttcccgccatctgatgagcagttgaaatctggaactgcctctgttgtgtgcctgctgaataacttctatcccagagaggccaaagtacagtggaaggtggataacgccctccaatcgggtaactcccaggagagtgtcacagagcaggacagcaaggacagcacctacagcctcagcagcaccctgacgctgagcaaagcagactacgagaaacacaaagtctacgcctgcgaagtcacccatcagggcctgagctcgcccgtcacaaagagcttcaacaggggagagtgttag

SEQ ID NO: 55 - DNA, 712 bp, synthetic construct
  misc_feature 1..712: note = nucleotides coding light chain of S53L conjuated with signal peptide
  source 1..712: mol_type = other DNA
atgggatggagctatatcatcctctttttggtggccacagcggccgatgtccactcgcagtctgtgctgactcagccaccctcagcgtctgggacccccgggcagagggtcaccatctcttgtactggctcttcatctaatattggcagtaattatgtctactggtaccagcagctcccaggaacggcccccaaactcctcatctatgctaatctgcatcggccaagcggggtccctgaccgattctctggctccaagtctggcacctcagcctccctggccatcagtgggctccggtccgaggatgaggctgattattactgtggtgcttgggatgatagcctgagtgcttatgtcttcgggggaggcaccaagctgacggtcctaagatctgtggctgcaccatctgtcttcatcttcccgccatctgatgagcagttgaaatctggaactgcctctgttgtgtgcctgctgaataacttctatcccagagaggccaaagtacagtggaaggtggataacgccctccaatcgggtaactcccaggagagtgtcacagagcaggacagcaaggacagcacctacagcctcagcagcaccctgacgctgagcaaagcagactacgagaaacacaaagtctacgcctgcgaagtcacccatcagggcctgagctcgcccgtcacaaagagcttcaacaggggagagtgttagv

SEQ ID NO: 56 - DNA, 711 bp, synthetic construct
  misc_feature 1..711: note = nucleotides coding light chain of S53T conjuated with signal peptide
  source 1..711: mol_type = other DNA
atgggatggagctatatcatcctctttttggtggccacagcggccgatgtccactcgcagtctgtgctgactcagccaccctcagcgtctgggacccccgggcagagggtcaccatctcttgtactggctcttcatctaatattggcagtaattatgtctactggtaccagcagctcccaggaacggcccccaaactcctcatctatgctaatactcatcggccaagcggggtccctgaccgattctctggctccaagtctggcacctcagcctccctggccatcagtgggctccggtccgaggatgaggctgattattactgtggtgcttgggatgatagcctgagtgcttatgtcttcgggggaggcaccaagctgacggtcctaagatctgtggctgcaccatctgtcttcatcttcccgccatctgatgagcagttgaaatctggaactgcctctgttgtgtgcctgctgaataacttctatcccagagaggccaaagtacagtggaaggtggataacgccctccaatcgggtaactcccaggagagtgtcacagagcaggacagcaaggacagcacctacagcctcagcagcaccctgacgctgagcaaagcagactacgagaaacacaaagtctacgcctgcgaagtcacccatcagggcctgagctcgcccgtcacaaagagcttcaacaggggagagtgttag

SEQ ID NO: 57 - DNA, 711 bp, synthetic construct
  misc_feature 1..711: note = nucleotides coding light chain of S53V conjuated with signal peptide
  source 1..711: mol_type = other DNA
atgggatggagctatatcatcctctttttggtggccacagcggccgatgtccactcgcagtctgtgctgactcagccaccctcagcgtctgggacccccgggcagagggtcaccatctcttgtactggctcttcatctaatattggcagtaattatgtctactggtaccagcagctcccaggaacggcccccaaactcctcatctatgctaatgtgcatcggccaagcggggtccctgaccgattctctggctccaagtctggcacctcagcctccctggccatcagtgggctccggtccgaggatgaggctgattattactgtggtgcttgggatgatagcctgagtgcttatgtcttcgggggaggcaccaagctgacggtcctaagatctgtggctgcaccatctgtcttcatcttcccgccatctgatgagcagttgaaatctggaactgcctctgttgtgtgcctgctgaataacttctatcccagagaggccaaagtacagtggaaggtggataacgccctccaatcgggtaactcccaggagagtgtcacagagcaggacagcaaggacagcacctacagcctcagcagcaccctgacgctgagcaaagcagactacgagaaacacaaagtctacgcctgcgaagtcacccatcagggcctgagctcgcccgtcacaaagagcttcaacaggggagagtgttag

SEQ ID NO: 58 - DNA, 711 bp, synthetic construct
  misc_feature 1..711: note = nucleotides coding light chain of S53Q conjuated with signal peptide
  source 1..711: mol_type = other DNA
atgggatggagctatatcatcctctttttggtggccacagcggccgatgtccactcgcagtctgtgctgactcagccaccctcagcgtctgggacccccgggcagagggtcaccatctcttgtactggctcttcatctaatattggcagtaattatgtctactggtaccagcagctcccaggaacggcccccaaactcctcatctatgctaatcagcatcggccaagcggggtccctgaccgattctctggctccaagtctggcacctcagcctccctggccatcagtgggctccggtccgaggatgaggctgattattactgtggtgcttgggatgatagcctgagtgcttatgtcttcgggggaggcaccaagctgacggtcctaagatctgtggctgcaccatctgtcttcatcttcccgccatctgatgagcagttgaaatctggaactgcctctgttgtgtgcctgctgaataacttctatcccagagaggccaaagtacagtggaaggtggataacgccctccaatcgggtaactcccaggagagtgtcacagagcaggacagcaaggacagcacctacagcctcagcagcaccctgacgctgagcaaagcagactacgagaaacacaaagtctacgcctgcgaagtcacccatcagggcctgagctcgcccgtcacaaagagcttcaacaggggagagtgttag

SEQ ID NO: 59 - DNA, 711 bp, synthetic construct
  misc_feature 1..711: note = nucleotides coding light chain of H54I conjuated with signal peptide
  source 1..711: mol_type = other DNA
atgggatggagctatatcatcctctttttggtggccacagcggccgatgtccactcgcagtctgtgctgactcagccaccctcagcgtctgggacccccgggcagagggtcaccatctcttgtactggctcttcatctaatattggcagtaattatgtctactggtaccagcagctcccaggaacggcccccaaactcctcatctatgctaatcagattcggccaagcggggtccctgaccgattctctggctccaagtctggcacctcagcctccctggccatcagtgggctccggtccgaggatgaggctgattattactgtggtgcttgggatgatagcctgagtgcttatgtcttcgggggaggcaccaagctgacggtcctaagatctgtggctgcaccatctgtcttcatcttcccgccatctgatgagcagttgaaatctggaactgcctctgttgtgtgcctgctgaataacttctatcccagagaggccaaagtacagtggaaggtggataacgccctccaatcgggtaactcccaggagagtgtcacagagcaggacagcaaggacagcacctacagcctcagcagcaccctgacgctgagcaaagcagactacgagaaacacaaagtctacgcctgcgaagtcacccatcagggcctgagctcgcccgtcacaaagagcttcaacaggggagagtgttag

SEQ ID NO: 60 - DNA, 711 bp, synthetic construct
  misc_feature 1..711: note = nucleotides coding light chain of H54L conjuated with signal peptide
  source 1..711: mol_type = other DNA
atgggatggagctatatcatcctctttttggtggccacagcggccgatgtccactcgcagtctgtgctgactcagccaccctcagcgtctgggacccccgggcagagggtcaccatctcttgtactggctcttcatctaatattggcagtaattatgtctactggtaccagcagctcccaggaacggcccccaaactcctcatctatgctaatcagcttcggccaagcggggtccctgaccgattctctggctccaagtctggcacctcagcctccctggccatcagtgggctccggtccgaggatgaggctgattattactgtggtgcttgggatgatagcctgagtgcttatgtcttcgggggaggcaccaagctgacggtcctaagatctgtggctgcaccatctgtcttcatcttcccgccatctgatgagcagttgaaatctggaactgcctctgttgtgtgcctgctgaataacttctatcccagagaggccaaagtacagtggaaggtggataacgccctccaatcgggtaactcccaggagagtgtcacagagcaggacagcaaggacagcacctacagcctcagcagcaccctgacgctgagcaaagcagactacgagaaacacaaagtctacgcctgcgaagtcacccatcagggcctgagctcgcccgtcacaaagagcttcaacaggggagagtgttag

SEQ ID NO: 61 - DNA, 711 bp, synthetic construct
  misc_feature 1..711: note = nucleotides coding light chain of H54K conjuated with signal peptide
  source 1..711: mol_type = other DNA
atgggatggagctatatcatcctctttttggtggccacagcggccgatgtccactcgcagtctgtgctgactcagccaccctcagcgtctgggacccccgggcagagggtcaccatctcttgtactggctcttcatctaatattggcagtaattatgtctactggtaccagcagctcccaggaacggcccccaaactcctcatctatgctaatcagaagcggccaagcggggtccctgaccgattctctggctccaagtctggcacctcagcctccctggccatcagtgggctccggtccgaggatgaggctgattattactgtggtgcttgggatgatagcctgagtgcttatgtcttcgggggaggcaccaagctgacggtcctaagatctgtggctgcaccatctgtcttcatcttcccgccatctgatgagcagttgaaatctggaactgcctctgttgtgtgcctgctgaataacttctatcccagagaggccaaagtacagtggaaggtggataacgccctccaatcgggtaactcccaggagagtgtcacagagcaggacagcaaggacagcacctacagcctcagcagcaccctgacgctgagcaaagcagactacgagaaacacaaagtctacgcctgcgaagtcacccatcagggcctgagctcgcccgtcacaaagagcttcaacaggggagagtgttag

SEQ ID NO: 62 - DNA, 711 bp, synthetic construct
  misc_feature 1..711: note = nucleotides coding light chain of H54Q conjuated with signal peptide
  source 1..711: mol_type = other DNA
atgggatggagctatatcatcctctttttggtggccacagcggccgatgtccactcgcagtctgtgctgactcagccaccctcagcgtctgggacccccgggcagagggtcaccatctcttgtactggctcttcatctaatattggcagtaattatgtctactggtaccagcagctcccaggaacggcccccaaactcctcatctatgctaatcagcaacggccaagcggggtccctgaccgattctctggctccaagtctggcacctcagcctccctggccatcagtgggctccggtccgaggatgaggctgattattactgtggtgcttgggatgatagcctgagtgcttatgtcttcgggggaggcaccaagctgacggtcctaagatctgtggctgcaccatctgtcttcatcttcccgccatctgatgagcagttgaaatctggaactgcctctgttgtgtgcctgctgaataacttctatcccagagaggccaaagtacagtggaaggtggataacgccctccaatcgggtaactcccaggagagtgtcacagagcaggacagcaaggacagcacctacagcctcagcagcaccctgacgctgagcaaagcagactacgagaaacacaaagtctacgcctgcgaagtcacccatcagggcctgagctcgcccgtcacaaagagcttcaacaggggagagtgttag

SEQ ID NO: 63 - DNA, 711 bp, synthetic construct
  misc_feature 1..711: note = nucleotides coding light chain of H54F conjuated with signal peptide
  source 1..711: mol_type = other DNA
atgggatggagctatatcatcctctttttggtggccacagcggccgatgtccactcgcagtctgtgctgactcagccaccctcagcgtctgggacccccgggcagagggtcaccatctcttgtactggctcttcatctaatattggcagtaattatgtctactggtaccagcagctcccaggaacggcccccaaactcctcatctatgctaatcagtttcggccaagcggggtccctgaccgattctctggctccaagtctggcacctcagcctccctggccatcagtgggctccggtccgaggatgaggctgattattactgtggtgcttgggatgatagcctgagtgcttatgtcttcgggggaggcaccaagctgacggtcctaagatctgtggctgcaccatctgtcttcatcttcccgccatctgatgagcagttgaaatctggaactgcctctgttgtgtgcctgctgaataacttctatcccagagaggccaaagtacagtggaaggtggataacgccctccaatcgggtaactcccaggagagtgtcacagagcaggacagcaaggacagcacctacagcctcagcagcaccctgacgctgagcaaagcagactacgagaaacacaaagtctacgcctgcgaagtcacccatcagggcctgagctcgcccgtcacaaagagcttcaacaggggagagtgttag

SEQ ID NO: 64 - DNA, 711 bp, synthetic construct
  misc_feature 1..711: note = nucleotides coding light chain of SH/IL conjuated with signal peptide
  source 1..711: mol_type = other DNA
atgggatggagctatatcatcctctttttggtggccacagcggccgatgtccactcgcagtctgtgctgactcagccaccctcagcgtctgggacccccgggcagagggtcaccatctcttgtactggctcttcatctaatattggcagtaattatgtctactggtaccagcagctcccaggaacggcccccaaactcctcatctatgctaatattcttcggccaagcggggtccctgaccgattctctggctccaagtctggcacctcagcctccctggccatcagtgggctccggtccgaggatgaggctgattattactgtggtgcttgggatgatagcctgagtgcttatgtcttcgggggaggcaccaagctgacggtcctaagatctgtggctgcaccatctgtcttcatcttcccgccatctgatgagcagttgaaatctggaactgcctctgttgtgtgcctgctgaataacttctatcccagagaggccaaagtacagtggaaggtggataacgccctccaatcgggtaactcccaggagagtgtcacagagcaggacagcaaggacagcacctacagcctcagcagcaccctgacgctgagcaaagcagactacgagaaacacaaagtctacgcctgcgaagtcacccatcagggcctgagctcgcccgtcacaaagagcttcaacaggggagagtgttag

SEQ ID NO: 65 - DNA, 711 bp, synthetic construct
  misc_feature 1..711: note = nucleotides coding light chain of SH/LL conjuated with signal peptide
  source 1..711: mol_type = other DNA
atgggatggagctatatcatcctctttttggtggccacagcggccgatgtccactcgcagtctgtgctgactcagccaccctcagcgtctgggacccccgggcagagggtcaccatctcttgtactggctcttcatctaatattggcagtaattatgtctactggtaccagcagctcccaggaacggcccccaaactcctcatctatgctaatctgcttcggccaagcggggtccctgaccgattctctggctccaagtctggcacctcagcctccctggccatcagtgggctccggtccgaggatgaggctgattattactgtggtgcttgggatgatagcctgagtgcttatgtcttcgggggaggcaccaagctgacggtcctaagatctgtggctgcaccatctgtcttcatcttcccgccatctgatgagcagttgaaatctggaactgcctctgttgtgtgcctgctgaataacttctatcccagagaggccaaagtacagtggaaggtggataacgccctccaatcgggtaactcccaggagagtgtcacagagcaggacagcaaggacagcacctacagcctcagcagcaccctgacgctgagcaaagcagactacgagaaacacaaagtctacgcctgcgaagtcacccatcagggcctgagctcgcccgtcacaaagagcttcaacaggggagagtgttag

SEQ ID NO: 66 - DNA, 711 bp, synthetic construct; identical to SEQ ID NO: 60
  misc_feature 1..711: note = nucleotides coding light chain of SH/QL conjuated with signal peptide
  source 1..711: mol_type = other DNA

SEQ ID NO: 67 - DNA, 711 bp, synthetic construct
  misc_feature 1..711: note = nucleotides coding light chain of SHL/ILN conjuated with signal peptide
  source 1..711: mol_type = other DNA
atgggatggagctatatcatcctctttttggtggccacagcggccgatgtccactcgcagtctgtgctgactcagccaccctcagcgtctgggacccccgggcagagggtcaccatctcttgtactggctcttcatctaatattggcagtaattatgtctactggtaccagcagctcccaggaacggcccccaaactcctcatctatgctaatattcttcggccaagcggggtccctgaccgattctctggctccaagtctggcacctcagcctccctggccatcagtgggctccggtccgaggatgaggctgattattactgtggtgcttgggatgatagcaatagtgcttatgtcttcgggggaggcaccaagctgacggtcctaagatctgtggctgcaccatctgtcttcatcttcccgccatctgatgagcagttgaaatctggaactgcctctgttgtgtgcctgctgaataacttctatcccagagaggccaaagtacagtggaaggtggataacgccctccaatcgggtaactcccaggagagtgtcacagagcaggacagcaaggacagcacctacagcctcagcagcaccctgacgctgagcaaagcagactacgagaaacacaaagtctacgcctgcgaagtcacccatcagggcctgagctcgcccgtcacaaagagcttcaacaggggagagtgttag

SEQ ID NO: 68 - DNA, 711 bp, synthetic construct
  misc_feature 1..711: note = nucleotides coding light chain of SHL/LLN conjuated with signal peptide
  source 1..711: mol_type = other DNA
atgggatggagctatatcatcctctttttggtggccacagcggccgatgtccactcgcagtctgtgctgactcagccaccctcagcgtctgggacccccgggcagagggtcaccatctcttgtactggctcttcatctaatattggcagtaattatgtctactggtaccagcagctcccaggaacggcccccaaactcctcatctatgctaatctgcttcggccaagcggggtccctgaccgattctctggctccaagtctggcacctcagcctccctggccatcagtgggctccggtccgaggatgaggctgattattactgtggtgcttgggatgatagcaatagtgcttatgtcttcgggggaggcaccaagctgacggtcctaagatctgtggctgcaccatctgtcttcatcttcccgccatctgatgagcagttgaaatctggaactgcctctgttgtgtgcctgctgaataacttctatcccagagaggccaaagtacagtggaaggtggataacgccctccaatcgggtaactcccaggagagtgtcacagagcaggacagcaaggacagcacctacagcctcagcagcaccctgacgctgagcaaagcagactacgagaaacacaaagtctacgcctgcgaagtcacccatcagggcctgagctcgcccgtcacaaagagcttcaacaggggagagtgttag

SEQ ID NO: 69 - DNA, 711 bp, synthetic construct
  misc_feature 1..711: note = nucleotides coding light chain of SHL/QLN conjuated with signal peptide
  source 1..711: mol_type = other DNA
atgggatggagctatatcatcctctttttggtggccacagcggccgatgtccactcgcagtctgtgctgactcagccaccctcagcgtctgggacccccgggcagagggtcaccatctcttgtactggctcttcatctaatattggcagtaattatgtctactggtaccagcagctcccaggaacggcccccaaactcctcatctatgctaatcagcttcggccaagcggggtccctgaccgattctctggctccaagtctggcacctcagcctccctggccatcagtgggctccggtccgaggatgaggctgattattactgtggtgcttgggatgatagcaatagtgcttatgtcttcgggggaggcaccaagctgacggtcctaagatctgtggctgcaccatctgtcttcatcttcccgccatctgatgagcagttgaaatctggaactgcctctgttgtgtgcctgctgaataacttctatcccagagaggccaaagtacagtggaaggtggataacgccctccaatcgggtaactcccaggagagtgtcacagagcaggacagcaaggacagcacctacagcctcagcagcaccctgacgctgagcaaagcagactacgagaaacacaaagtctacgcctgcgaagtcacccatcagggcctgagctcgcccgtcacaaagagcttcaacaggggagagtgttag

SEQ ID NO: 70 - DNA, 21 bp, synthetic construct
  misc_feature 1..21: note = nucleotides coding ANSHRPS
  source 1..21: mol_type = other DNA
gctaatagtcatcggccaagc

SEQ ID NO: 71 - DNA, 33 bp, synthetic construct
  misc_feature 1..33: note = nucleotides coding GAWDDSLSAY
  source 1..33: mol_type = other DNA
ggtgcttgggatgatagcctgagtgcttatgtc

SEQ ID NO: 72 - DNA, 26 bp, synthetic construct
  misc_feature 1..26: note = Forward primer of CDR2 for variable region in light chain of S53I
  source 1..26: mol_type = other DNA
ctaatattcatcggccaagcggggtc

SEQ ID NO: 73 - DNA, 34 bp, synthetic construct
  misc_feature 1..34: note = Reverse primer of CDR2 for variable region in light chain of S53I
  source 1..34: mol_type = other DNA
gccgatgaatattagcatagatgaggagtttggg

SEQ ID NO: 74 - DNA, 26 bp, synthetic construct
  misc_feature 1..26: note = Forward primer of CDR2 for variable region in light chain of S53L
  source 1..26: mol_type = other DNA
ctaatctgcatcggccaagcggggtc

SEQ ID NO: 75 - DNA, 34 bp, synthetic construct
  misc_feature 1..34: note = Reverse primer of CDR2 for variable region in light chain of S53L
  source 1..34: mol_type = other DNA
gccgatgcagattagcatagatgaggagtttggg

SEQ ID NO: 76 - DNA, 26 bp, synthetic construct
  misc_feature 1..26: note = Forward primer of CDR2 for variable region in light chain of S53T
  source 1..26: mol_type = other DNA
ctaatactcatcggccaagcggggtc

SEQ ID NO: 77 - DNA, 34 bp, synthetic construct
  misc_feature 1..34: note = Reverse primer of CDR2 for variable region in light chain of S53T
  source 1..34: mol_type = other DNA
gccgatgagtattagcatagatgaggagtttggg

SEQ ID NO: 78 - DNA, 26 bp, synthetic construct
  misc_feature 1..26: note = Forward primer of CDR2 for variable region in light chain of S53V
  source 1..26: mol_type = other DNA
ctaatgtgcatcggccaagcggggtc

SEQ ID NO: 79 - DNA, 34 bp, synthetic construct
  misc_feature 1..34: note = Reverse primer of CDR2 for variable region in light chain of S53V
  source 1..34: mol_type = other DNA
gccgatgcacattagcatagatgaggagtttggg

SEQ ID NO: 80 - DNA, 26 bp, synthetic construct
  misc_feature 1..26: note = Forward primer of CDR2 for variable region in light chain of S53Q
  source 1..26: mol_type = other DNA
ctaatcagcatcggccaagcggggtc

SEQ ID NO: 81 - DNA, 34 bp, synthetic construct
  misc_feature 1..34: note = Reverse primer of CDR2 for variable region in light chain of S53Q
  source 1..34: mol_type = other DNA
gccgatgctgattagcatagatgaggagtttggg

SEQ ID NO: 82 - DNA, 28 bp, synthetic construct
  misc_feature 1..28: note = Forward primer of CDR2 for variable region in light chain of H54I
  source 1..28: mol_type = other DNA
gctaatagtattcggccaagcggggtcc

SEQ ID NO: 83 - DNA, 33 bp, synthetic construct
  misc_feature 1..33: note = Reverse primer of CDR2 for variable region in light chain of H54I
  source 1..33: mol_type = other DNA
ccgaatactattagcatagatgaggagtttggg

SEQ ID NO: 84 - DNA, 28 bp, synthetic construct
  misc_feature 1..28: note = Forward primer of CDR2 for variable region in light chain of H54L
  source 1..28: mol_type = other DNA
gctaatagtcttcggccaagcggggtcc

SEQ ID NO: 85 - DNA, 28 bp, synthetic construct
  misc_feature 1..28: note = Reverse primer of CDR2 for variable region in light chain of H54L
  source 1..28: mol_type = other DNA
gctaatagtcttcggccaagcggggtcc

SEQ ID NO: 86 - DNA, 28 bp, synthetic construct
  misc_feature 1..28: note = Forward primer of CDR2 for variable region in light chain of H54K
  source 1..28: mol_type = other DNA
gctaatagtaagcggccaagcggggtcc

SEQ ID NO: 87 - DNA, 33 bp, synthetic construct
  misc_feature 1..33: note = Reverse primer of CDR2 for variable region in light chain of H54K
  source 1..33: mol_type = other DNA
ccgcttactattagcatagatgaggagtttggg

SEQ ID NO: 88 - DNA, 28 bp, synthetic construct
  misc_feature 1..28: note = Forward primer of CDR2 for variable region in light chain of H54E
  source 1..28: mol_type = other DNA
gctaatagtcgaaggccaagcggggtcc

SEQ ID NO: 89 - DNA, 33 bp, synthetic construct
  misc_feature 1..33: note = Reverse primer of CDR2 for variable region in light chain of H54E
  source 1..33: mol_type = other DNA
ccgttcactattagcatagatgaggagtttggg

SEQ ID NO: 90 - DNA, 28 bp, synthetic construct
  misc_feature 1..28: note = Forward primer of CDR2 for variable region in light chain of H54F
  source 1..28: mol_type = other DNA
gctaatagttttcggccaagcggggtcc

SEQ ID NO: 91 - DNA, 33 bp, synthetic construct
  misc_feature 1..33: note = Reverse primer of CDR2 for variable region in light chain of H54F
  source 1..33: mol_type = other DNA
ccgaaaactattagcatagatgaggagtttggg

SEQ ID NO: 92 - DNA, 30 bp, synthetic construct
  misc_feature 1..30: note = Forward primer of CDR3 for variable region in light chain
  source 1..30: mol_type = other DNA
gatagcaatagtgcttatgtcttcggggga

SEQ ID NO: 93 - DNA, 29 bp, synthetic construct
  misc_feature 1..29: note = Reverse primer of CDR3 for variable region in light chain
  source 1..29: mol_type = other DNA
aagcactattgctatcatcccaagcacca

SEQ ID NO: 94 - protein, 471 aa, synthetic construct
  REGION 1..471: note = human WARS1
MPNSEPASLLELFNSIATQGELVRSLKAGNASKDEIDSAVKMLVSLKMSYKAAAGEDYKADCPPGNPAPTSNHGPDATEAEEDFVDPWTVQTSSAKGIDYDKLIVRFGSSKIDKELINRIERATGQRPHHFLRRGIFFSHRDMNQVLDAYENKKPFYLYTGRGPSSEAMHVGHLIPFIFTKWLQDVFNVPLVIQMTDDEKYLWKDLTLDQAYSYAVENAKDIIACGFDINKTFIFSDLDYMGMSSGFYKNVVKIQKHVTFNQVKGIFGFTDSDCIGKISFPAIQAAPSFSNSFPQIFRDRTDIQCLIPCAIDQDPYFRMTRDVAPRIGYPKPALLHSTFFPALQGAQTKMSASDPNSSIFLTDTAKQIKTKVNKHAFSGGRDTIEEHRQFGGNCDVDVSFMYLTFFLEDDDKLEQIRKDYTSGAMLTGELKKALIEVLQPLIAEHQARRKEVTDEIVKEFMTPRKLSFDFQ

SEQ ID NO: 95 - protein, 8 aa, synthetic construct
  REGION 1..8: note = L-CDR2 of variable region in light chain for anti-WARS1 antibody
  VARIANT 3: note = X can be Ala, Val, Ile, Leu, Met, Phe, Tyr, Trp, Lys, Arg, His, Asp, Ser, Thr, Glu, Asn, Gln, Cys, Gly or Pro
  VARIANT 4: note = X can be Ala, Val, Ile, Leu, Met, Phe, Tyr, Trp, Lys, Arg, His, Asp, Ser, Thr, Glu, Asn, Gln, Cys, Gly or Pro
  VARIANT 3..4: note = When X of the third amino acid is Ser, X of the fourth amino acid is not His
ANXXHRPS

SEQ ID NO: 96 - protein, 11 aa, synthetic construct
  REGION 1..11: note = L-CDR3 of variable region in light chain for anti-WARS1 antibody
  VARIANT 7: note = X can be Ala, Val, Ile, Leu, Met, Phe, Tyr, Trp, Lys, Arg, His, Asp, Ser, Thr, Glu, Asn, Gln, Cys, Gly or Pro
GAWDDSXSAYV

SEQ ID NO: 97 - protein, 236 aa, synthetic construct
  REGION 1..236: note = light chain of GKB101 conjuated with signal peptide
MGWSYIILFLVATAADVHSQSVLTQPPSASGTPGQRVTISCTGSSSNIGSNYVYWYQQLPGTAPKLLIYANSHRPSGVPDRFSGSKSGTSASLAISGLRSEDEADYYCGAWDDSLSAYVFGGGTKLTVLRSVAAPSVFIFPPSDEQLKSGTASVVCLLNNFYPREAKVQWKVDNALQSGNSQESVTEQDSKDSTYSLSSTLTLSKADYEKHKVYACEVTHQGLSSPVTKSFNRGEC

SEQ ID NO: 98 - protein, 236 aa, synthetic construct
  REGION 1..236: note = light chain of S53I conjuated with signal peptide
MGWSYIILFLVATAADVHSQSVLTQPPSASGTPGQRVTISCTGSSSNIGSNYVYWYQQLPGTAPKLLIYANIHRPSGVPDRFSGSKSGTSASLAISGLRSEDEADYYCGAWDDSLSAYVFGGGTKLTVLRSVAAPSVFIFPPSDEQLKSGTASVVCLLNNFYPREAKVQWKVDNALQSGNSQESVTEQDSKDSTYSLSSTLTLSKADYEKHKVYACEVTHQGLSSPVTKSFNRGEC

SEQ ID NO: 99 - protein, 236 aa, synthetic construct
  REGION 1..236: note = light chain of S53L conjuated with signal peptide
MGWSYIILFLVATAADVHSQSVLTQPPSASGTPGQRVTISCTGSSSNIGSNYVYWYQQLPGTAPKLLIYANLHRPSGVPDRFSGSKSGTSASLAISGLRSEDEADYYCGAWDDSLSAYVFGGGTKLTVLRSVAAPSVFIFPPSDEQLKSGTASVVCLLNNFYPREAKVQWKVDNALQSGNSQESVTEQDSKDSTYSLSSTLTLSKADYEKHKVYACEVTHQGLSSPVTKSFNRGEC

SEQ ID NO: 100 - protein, 236 aa, synthetic construct
  REGION 1..236: note = light chain of S53T conjuated with signal peptide
MGWSYIILFLVATAADVHSQSVLTQPPSASGTPGQRVTISCTGSSSNIGSNYVYWYQQLPGTAPKLLIYANTHRPSGVPDRFSGSKSGTSASLAISGLRSEDEADYYCGAWDDSLSAYVFGGGTKLTVLRSVAAPSVFIFPPSDEQLKSGTASVVCLLNNFYPREAKVQWKVDNALQSGNSQESVTEQDSKDSTYSLSSTLTLSKADYEKHKVYACEVTHQGLSSPVTKSFNRGEC

SEQ ID NO: 101 - protein, 236 aa, synthetic construct
  REGION 1..236: note = light chain of S53V conjuated with signal peptide
MGWSYIILFLVATAADVHSQSVLTQPPSASGTPGQRVTISCTGSSSNIGSNYVYWYQQLPGTAPKLLIYANVHRPSGVPDRFSGSKSGTSASLAISGLRSEDEADYYCGAWDDSLSAYVFGGGTKLTVLRSVAAPSVFIFPPSDEQLKSGTASVVCLLNNFYPREAKVQWKVDNALQSGNSQESVTEQDSKDSTYSLSSTLTLSKADYEKHKVYACEVTHQGLSSPVTKSFNRGEC

SEQ ID NO: 102 - protein, 236 aa, synthetic construct
  REGION 1..236: note = light chain of S53Q conjuated with signal peptide
MGWSYIILFLVATAADVHSQSVLTQPPSASGTPGQRVTISCTGSSSNIGSNYVYWYQQLPGTAPKLLIYANQHRPSGVPDRFSGSKSGTSASLAISGLRSEDEADYYCGAWDDSLSAYVFGGGTKLTVLRSVAAPSVFIFPPSDEQLKSGTASVVCLLNNFYPREAKVQWKVDNALQSGNSQESVTEQDSKDSTYSLSSTLTLSKADYEKHKVYACEVTHQGLSSPVTKSFNRGEC

SEQ ID NO: 103 - protein, 236 aa, synthetic construct
  REGION 1..236: note = light chain of H54I conjuated with signal peptide
MGWSYIILFLVATAADVHSQSVLTQPPSASGTPGQRVTISCTGSSSNIGSNYVYWYQQLPGTAPKLLIYANQIRPSGVPDRFSGSKSGTSASLAISGLRSEDEADYYCGAWDDSLSAYVFGGGTKLTVLRSVAAPSVFIFPPSDEQLKSGTASVVCLLNNFYPREAKVQWKVDNALQSGNSQESVTEQDSKDSTYSLSSTLTLSKADYEKHKVYACEVTHQGLSSPVTKSFNRGEC

SEQ ID NO: 104 - protein, 236 aa, synthetic construct
  REGION 1..236: note = light chain of H54L conjuated with signal peptide
MGWSYIILFLVATAADVHSQSVLTQPPSASGTPGQRVTISCTGSSSNIGSNYVYWYQQLPGTAPKLLIYANQLRPSGVPDRFSGSKSGTSASLAISGLRSEDEADYYCGAWDDSLSAYVFGGGTKLTVLRSVAAPSVFIFPPSDEQLKSGTASVVCLLNNFYPREAKVQWKVDNALQSGNSQESVTEQDSKDSTYSLSSTLTLSKADYEKHKVYACEVTHQGLSSPVTKSFNRGEC

SEQ ID NO: 105 - protein, 236 aa, synthetic construct
  REGION 1..236: note = light chain of H54K conjuated with signal peptide
MGWSYIILFLVATAADVHSQSVLTQPPSASGTPGQRVTISCTGSSSNIGSNYVYWYQQLPGTAPKLLIYANQKRPSGVPDRFSGSKSGTSASLAISGLRSEDEADYYCGAWDDSLSAYVFGGGTKLTVLRSVAAPSVFIFPPSDEQLKSGTASVVCLLNNFYPREAKVQWKVDNALQSGNSQESVTEQDSKDSTYSLSSTLTLSKADYEKHKVYACEVTHQGLSSPVTKSFNRGEC

SEQ ID NO: 106 - protein, 236 aa, synthetic construct
  REGION 1..236: note = light chain of H54Q conjuated with signal peptide
MGWSYIILFLVATAADVHSQSVLTQPPSASGTPGQRVTISCTGSSSNIGSNYVYWYQQLPGTAPKLLIYANQQRPSGVPDRFSGSKSGTSASLAISGLRSEDEADYYCGAWDDSLSAYVFGGGTKLTVLRSVAAPSVFIFPPSDEQLKSGTASVVCLLNNFYPREAKVQWKVDNALQSGNSQESVTEQDSKDSTYSLSSTLTLSKADYEKHKVYACEVTHQGLSSPVTKSFNRGEC

SEQ ID NO: 107 - protein, 236 aa, synthetic construct
  REGION 1..236: note = light chain of H54F conjuated with signal peptide
MGWSYIILFLVATAADVHSQSVLTQPPSASGTPGQRVTISCTGSSSNIGSNYVYWYQQLPGTAPKLLIYANQFRPSGVPDRFSGSKSGTSASLAISGLRSEDEADYYCGAWDDSLSAYVFGGGTKLTVLRSVAAPSVFIFPPSDEQLKSGTASVVCLLNNFYPREAKVQWKVDNALQSGNSQESVTEQDSKDSTYSLSSTLTLSKADYEKHKVYACEVTHQGLSSPVTKSFNRGEC

SEQ ID NO: 108 - protein, 236 aa, synthetic construct
  REGION 1..236: note = light chain of SH/IL conjuated with signal peptide
MGWSYIILFLVATAADVHSQSVLTQPPSASGTPGQRVTISCTGSSSNIGSNYVYWYQQLPGTAPKLLIYANILRPSGVPDRFSGSKSGTSASLAISGLRSEDEADYYCGAWDDSLSAYVFGGGTKLTVLRSVAAPSVFIFPPSDEQLKSGTASVVCLLNNFYPREAKVQWKVDNALQSGNSQESVTEQDSKDSTYSLSSTLTLSKADYEKHKVYACEVTHQGLSSPVTKSFNRGEC

SEQ ID NO: 109 - protein, 236 aa, synthetic construct
  REGION 1..236: note = light chain of SH/LL conjuated with signal peptide
MGWSYIILFLVATAADVHSQSVLTQPPSASGTPGQRVTISCTGSSSNIGSNYVYWYQQLPGTAPKLLIYANLLRPSGVPDRFSGSKSGTSASLAISGLRSEDEADYYCGAWDDSLSAYVFGGGTKLTVLRSVAAPSVFIFPPSDEQLKSGTASVVCLLNNFYPREAKVQWKVDNALQSGNSQESVTEQDSKDSTYSLSSTLTLSKADYEKHKVYACEVTHQGLSSPVTKSFNRGEC

SEQ ID NO: 110 - protein, 236 aa, synthetic construct; identical to SEQ ID NO: 104
  REGION 1..236: note = light chain of SH/QL conjuated with signal peptide

SEQ ID NO: 111 - protein, 236 aa, synthetic construct
  REGION 1..236: note = light chain of SHL/ILN conjuated with signal peptide
MGWSYIILFLVATAADVHSQSVLTQPPSASGTPGQRVTISCTGSSSNIGSNYVYWYQQLPGTAPKLLIYANILRPSGVPDRFSGSKSGTSASLAISGLRSEDEADYYCGAWDDSNSAYVFGGGTKLTVLRSVAAPSVFIFPPSDEQLKSGTASVVCLLNNFYPREAKVQWKVDNALQSGNSQESVTEQDSKDSTYSLSSTLTLSKADYEKHKVYACEVTHQGLSSPVTKSFNRGEC

SEQ ID NO: 112 - protein, 236 aa, synthetic construct
  REGION 1..236: note = light chain of SHL/LLN conjuated with signal peptide
MGWSYIILFLVATAADVHSQSVLTQPPSASGTPGQRVTISCTGSSSNIGSNYVYWYQQLPGTAPKLLIYANLLRPSGVPDRFSGSKSGTSASLAISGLRSEDEADYYCGAWDDSNSAYVFGGGTKLTVLRSVAAPSVFIFPPSDEQLKSGTASVVCLLNNFYPREAKVQWKVDNALQSGNSQESVTEQDSKDSTYSLSSTLTLSKADYEKHKVYACEVTHQGLSSPVTKSFNRGEC

SEQ ID NO: 113 - protein, 236 aa, synthetic construct
  REGION 1..236: note = light chain of SHL/QLN conjuated with signal peptide
MGWSYIILFLVATAADVHSQSVLTQPPSASGTPGQRVTISCTGSSSNIGSNYVYWYQQLPGTAPKLLIYANQLRPSGVPDRFSGSKSGTSASLAISGLRSEDEADYYCGAWDDSNSAYVFGGGTKLTVLRSVAAPSVFIFPPSDEQLKSGTASVVCLLNNFYPREAKVQWKVDNALQSGNSQESVTEQDSKDSTYSLSSTLTLSKADYEKHKVYACEVTHQGLSSPVTKSFNRGEC

SEQ ID NO: 114 - DNA, 4402 bp, synthetic construct
  misc_feature 1..4402: note = pOptiVec Topo vector
  source 1..4402: mol_type = other DNA
aaagtgccacctgacgtcgacggatcgggagatcagttgacattgattattgactagttattaatagtaatcaattacggggtcattagttcatagcccatatatggagttccgcgttacataacttacggtaaatggcccgcctggctgaccgcccaacgacccccgcccattgacgtcaataatgacgtatgttcccatagtaacgccaatagggactttccattgacgtcaatgggtggagtatttacggtaaactgcccacttggcagtacatcaagtgtatcatatgccaagtacgccccctattgacgtcaatgacggtaaatggcccgcctggcattatgcccagtacatgaccttatgggactttcctacttggcagtacatctacgtattagtcatcgctattaccatggtgatgcggttttggcagtacatcaatgggcgtggatagcggtttgactcacggggatttccaagtctccaccccattgacgtcaatgggagtttgttttggcaccaaaatcaacgggactttccaaaatgtcgtaacaactccgccccattgacgcaaatgggcggtaggcgtgtacggtgggaggtctatataagcagagctcgtttagtgaaccgtcagatcgcctggagacgccatccacgctgttttgacctccatagaagacaccgggaccgatccagcctccggactctagaggatccaacccttaagggttggatccctaccggtgctgcggccgcgcagttaacgccgcccctctccctcccccccccctaacgttactggccgaagccgcttggaataaggccggtgtgcgtttgtctatatgttattttccaccatattgccgtcttttggcaatgtgagggcccggaaacctggccctgtcttcttgacgagcattcctaggggtctttcccctctcgccaaaggaatgcaaggtctgttgaatgtcgtgaaggaagcagttcctctggaagcttcttgaagacaaacaacgtctgtagcgaccctttgcaggcagcggaaccccccacctggcgacaggtgcctctgcggccaaaagccacgtgtataagatacacctgcaaaggcggcacaaccccagtgccacgttgtgagttggatagttgtggaaagagtcaaatggctctcctcaagcgtattcaacaaggggctgaaggatgcccagaaggtaccccattgtatgggatctgatctggggcctcggtacacatgctttacatgtgtttagtcgaggttaaaaaaacgtctaggccccccgaaccacggggacgtggttttcctttgaaaaacacgatgataatatggccacaagatctgccaccatggttcgaccattgaactgcatcgtcgccgtgtcccaaaatatggggattggcaagaacggagacctaccctggcctccgctcaggaacgagttcaagtacttccaaagaatgaccacaacctcttcagtggaaggtaaacagaatctggtgattatgggtaggaaaacctggttctccattcctgagaagaatcgacctttaaaggacagaattaatatagttctcagtagagaactcaaagaaccaccacgaggagctcattttcttgccaaaagtttggatgatgccttaagacttattgaacaaccggaattggcaagtaaagtagacatggtttggatagtcggaggcagttctgtttaccaggaagccatgaatcaaccaggccacctcagactctttgtgacaaggatcatgcaggaatttgaaagtgacacgtttttcccagaaattgatttggggaaatataaacttctcccagaatacccaggcgtcctctctgaggtccaggaggaaaaaggcatcaagtataagtttgaagtctacgagaagaaagactaaaaccggttagtaatgagtttaaacgggggaggctaactgaaacacggaaggagacaataccggaaggaacccgcgctatgacggcaataaaaagacagaataaaacgcacgggtgttgggtcgtttgttcataaacgcggggttcggtcccagggctggcactctgtcgataccccaccgagaccccattggggccaatacgcccgcgtttcttccttttccccaccccaccccccaagttcgggtgaaggcccagggctcgcagccaacgtcggggcggcaggccctgccattaccgtcgacctctagctagagcttggcgtaatcatggtcatagctgtttcctgtgtgaaattgttatccgctcacaattccacacaacatacgagccggaagcataaagtgtaaagcctggggtgcctaatgagtgagctaactcacattaattgcgttgcgctcactgcccgctttccagtcgggaaacctgtcgtgccagctgcattaatgaatcggccaacgcgcggggagaggcggtttgcgtattgggcgctcttccgcttcctcgctcactgactcgctgcgctcggtcgttcggctgcggcgagcggtatcagctcactcaaaggcggtaatacggttatccacagaatcaggggataacgcaggaaagaacatgtgagcaaaaggccagcaaaaggccaggaaccgtaaaaaggccgcgttgctggcgtttttccataggctccgcccccctgacgagcatcacaaaaatcgacgctcaagtcagaggtggcgaaacccgacaggactataaagataccaggcgtttccccctggaagctccctcgtgcgctctcctgttccgaccctgccgcttaccggatacctgtccgcctttctcccttcgggaagcgtggcgctttctcatagctcacgctgtaggtatctcagttcggtgtaggtcgttcgctccaagctgggctgtgtgcacgaaccccccgttcagcccgaccgctgcgccttatccggtaactatcgtcttgagtccaacccggtaagacacgacttatcgccactggcagcagccactggtaacaggattagcagagcgaggtatgtaggcggtgctacagagttcttgaagtggtggcctaactacggctacactagaagaacagtatttggtatctgcgctctgctgaagccagttaccttcggaaaaagagttggtagctcttgatccggcaaacaaaccaccgctggtagcggtttttttgtttgcaagcagcagattacgcgcagaaaaaaaggatctcaagaagatcctttgatcttttctacggggtctgacgctcagtggaacgaaaactcacgttaagggattttggtcatgagattatcaaaaaggatcttcacctagatccttttaaattaaaaatgaagttttaaatcaatctaaagtatatatgagtaaacttggtctgacagttaccaatgcttaatcagtgaggcacctatctcagcgatctgtctatttcgttcatccatagttgcctgactccccgtcgtgtagataactacgatacgggagggcttaccatctggccccagtgctgcaatgataccgcgagacccacgctcaccggctccagatttatcagcaataaaccagccagccggaagggccgagcgcagaagtggtcctgcaactttatccgcctccatccagtctattaattgttgccgggaagctagagtaagtagttcgccagttaatagtttgcgcaacgttgttgccattgctacaggcatcgtggtgtcacgctcgtcgtttggtatggcttcattcagctccggttcccaacgatcaaggcgagttacatgatcccccatgttgtgcaaaaaagcggttagctccttcggtcctccgatcgttgtcagaagtaagttggccgcagtgttatcactcatggttatggcagcactgcataattctcttactgtcatgccatccgtaagatgcttttctgtgactggtgagtactcaaccaagtcattctgagaatagtgtatgcggcgaccgagttgctcttgcccggcgtcaatacgggataataccgcgccacatagcagaactttaaaagtgctcatcattggaaaacgttcttcggggcgaaaactctcaaggatcttaccgctgttgagatccagttcgatgtaacccactcgtgcacccaactgatcttcagcatcttttactttcaccagcgtttctgggtgagcaaaaacaggaaggcaaaatgccgcaaaaaagggaataagggcgacacggaaatgttgaatactcatactcttcctttttcaatattattgaagcatttatcagggttattgtctcatgagcggatacatatttgaatgtatttagaaaaataaacaaataggggttccgcgcacatttccccga

SEQ ID NO: 115 - protein, 70 aa, synthetic construct
  REGION 1..70: note = P23381 human WARS1 N-terminal sequence involved WHEP domain
MPNSEPASLLELFNSIATQGELVRSLKAGNASKDEIDSAVKMLVSLKMSYKAAAGEDYKADCPPGNPAPT

SEQ ID NO: 116 - protein, 70 aa, synthetic construct
  REGION 1..70: note = P32921 Mouse WARS1 N-terminal sequence involved WHEP domain
PSGESCTSPLELFNSIATQGELVRSLKAGNAPKDEIDSAVKMLLSLKMSYKAAMGEEYKAGCPPGNPTAG

SEQ ID NO: 117 - protein, 70 aa, synthetic construct
  REGION 1..70: note = marmoset WARS1 N-terminal sequence involved WHEP domain
ANSEACASPLELFNSVTTQGEHVRALKAGNASKDEIDSAVKMLLSLKMSYKAAMGEDYKANCPPGSLAPS

SEQ ID NO: 118 - DNA, 20 bp, synthetic construct
  source 1..20: mol_type = other DNA
  misc_feature 1..20: note = FOXP3_F
cctgccttggtacattcgtg

SEQ ID NO: 119 - DNA, 20 bp, synthetic construct
  source 1..20: mol_type = other DNA
  misc_feature 1..20: note = FOXP3_R
tgttgtgggtgagtgctttg

SEQ ID NO: 120 - DNA, 20 bp, synthetic construct
  source 1..20: mol_type = other DNA
  misc_feature 1..20: note = IFNgamma_F
acagctctccgtcctcgtat

SEQ ID NO: 121 - DNA, 19 bp, synthetic construct
  source 1..19: mol_type = other DNA
  misc_feature 1..19: note = IFNgamma_R
ccttagagtagaaagaccg

SEQ ID NO: 122 - DNA, 20 bp, synthetic construct
  source 1..20: mol_type = other DNA
  misc_feature 1..20: note = IL-6_F
cctctggtcttctggagtac

SEQ ID NO: 123 - DNA, 19 bp, synthetic construct
  source 1..19: mol_type = other DNA
  misc_feature 1..19: note = IL-6_R
ggaaattggggtaggaagg

SEQ ID NO: 124 - DNA, 19 bp, synthetic construct
  source 1..19: mol_type = other DNA
  misc_feature 1..19: note = IL-10_F
agccacatgctcctagagc

SEQ ID NO: 125 - DNA, 20 bp, synthetic construct
  source 1..20: mol_type = other DNA
  misc_feature 1..20: note = IL-10_R
gcctggggcatcacttctac

SEQ ID NO: 126 - DNA, 22 bp, synthetic construct
  source 1..22: mol_type = other DNA
  misc_feature 1..22: note = iNOS_F
ggagcctttagacctcaacaga

SEQ ID NO: 127 - DNA, 18 bp, synthetic construct
  source 1..18: mol_type = other DNA
  misc_feature 1..18: note = iNOS_R
tgaacgaggagggtggtg

SEQ ID NO: 128 - DNA, 20 bp, synthetic construct
  source 1..20: mol_type = other DNA
  misc_feature 1..20: note = MCP-1_F
gggacgtttgctatgatgcc

SEQ ID NO: 129 - DNA, 24 bp, synthetic construct
  source 1..24: mol_type = other DNA
  misc_feature 1..24: note = MCP-1_R
cctactcattgggatactcttgct

SEQ ID NO: 130 - DNA, 20 bp, synthetic construct
  source 1..20: mol_type = other DNA
  misc_feature 1..20: note = TGF-beta1_F
accatgccaacttctgtctg

SEQ ID NO: 131 - DNA, 20 bp, synthetic construct
  source 1..20: mol_type = other DNA
  misc_feature 1..20: note = TFG-beta1_R
cgggttgtgttggttgtaga

SEQ ID NO: 132 - DNA, 20 bp, synthetic construct
  source 1..20: mol_type = other DNA
  misc_feature 1..20: note = TNF-alpha_F
gcctcttctcattcctgctt

SEQ ID NO: 133 - DNA, 21 bp, synthetic construct
  source 1..21: mol_type = other DNA
  misc_feature 1..21: note = TNF-alpha_R
tgggaacttctcatccctttg

SEQ ID NO: 134 - DNA, 20 bp, synthetic construct
  source 1..20: mol_type = other DNA
  misc_feature 1..20: note = WARS1_F
caggatgtgttcaatgtgcc

SEQ ID NO: 135 - DNA, 20 bp, synthetic construct
  source 1..20: mol_type = other DNA
  misc_feature 1..20: note = WARS1_R
ttgaaggtgacgtgcttctg

SEQ ID NO: 136 - DNA, 24 bp, synthetic construct
  source 1..24: mol_type = other DNA
  misc_feature 1..24: note = GAPDH_F
tcaacagcaactcccactcttcca

SEQ ID NO: 137 - DNA, 24 bp, synthetic construct
  source 1..24: mol_type = other DNA
  misc_feature 1..24: note = GAPDH_R
accctgttgctgtagccgtattca

SEQ ID NO: 138 - DNA, 21 bp, synthetic construct
  source 1..21: mol_type = other DNA
  misc_feature 1..21: note = IFN-gamma_F
gaactggcaaaaggatggtga

SEQ ID NO: 139 - DNA, 21 bp, synthetic construct
  source 1..21: mol_type = other DNA
  misc_feature 1..21: note = IFN-gamm_R
tgtgggttgttgacctcaaac

SEQ ID NO: 140 - DNA, 22 bp, synthetic construct
  source 1..22: mol_type = other DNA
  misc_feature 1..22: note = IL-6_F
taccacttcacaagtcggaggc

SEQ ID NO: 141 - DNA, 20 bp, synthetic construct
  source 1..20: mol_type = other DNA
  misc_feature 1..20: note = IL-6_R
ctgcaagtgcatcgttgttc

SEQ ID NO: 142 - DNA, 22 bp, synthetic construct
  source 1..22: mol_type = other DNA
  misc_feature 1..22: note = TNF-alpha_F
ggtgcctatgtctcagcctctt

SEQ ID NO: 143 - DNA, 23 bp, synthetic construct
  source 1..23: mol_type = other DNA
  misc_feature 1..23: note = TNF-alpha_R
gccatagaactgatgagagggag

SEQ ID NO: 144 - DNA, 22 bp, synthetic construct
  source 1..22: mol_type = other DNA
  misc_feature 1..22: note = CXCL9_F
atgaagtccgctgttcttttcc

SEQ ID NO: 145 - DNA, 22 bp, synthetic construct
  source 1..22: mol_type = other DNA
  misc_feature 1..22: note = CXCL9_R
gtctcttatgtagtcttccttg

SEQ ID NO: 146 - DNA, 24 bp, synthetic construct
  source 1..24: mol_type = other DNA
  misc_feature 1..24: note = MUC5AC_F
agaatatctttcaggacccctgct

SEQ ID NO: 147 - DNA, 23 bp, synthetic construct
  source 1..23: mol_type = other DNA
  misc_feature 1..23: note = MUC5AC_R
acaccagtgctgagcatactttt

SEQ ID NO: 148 - DNA, 20 bp, synthetic construct
  source 1..20: mol_type = other DNA
  misc_feature 1..20: note = TARC_F
tccagggcaagctcatctgt

SEQ ID NO: 149 - DNA, 20 bp, synthetic construct
  source 1..20: mol_type = other DNA
  misc_feature 1..20: note = TARC_R
aatgcctcagcgggaaggtc

SEQ ID NO: 150 - DNA, 16 bp, synthetic construct
  source 1..16: mol_type = other DNA
  misc_feature 1..16: note = TRPA1_F
tgagatcgaccggagt

SEQ ID NO: 151 - DNA, 15 bp, synthetic construct
  source 1..15: mol_type = other DNA
  misc_feature 1..15: note = TRPA1_R
tgctgaaggcatctt

SEQ ID NO: 152 - DNA, 16 bp, synthetic construct
  source 1..16: mol_type = other DNA
  misc_feature 1..16: note = Eotaxin_F
tgctgaaggcatcttg

SEQ ID NO: 153 - DNA, 20 bp, synthetic construct
  source 1..20: mol_type = other DNA
  misc_feature 1..20: note = Eotoxin_R
aatatcagcaccagtcgccc